European Patent Specification EP 3 448 419 B1, published June 7, 2023. Title: INTERFERON BETA ANTIBODIES AND USES THEREOF. Applicant: PFIZER INC. THE BRIGHAM AND WOMEN'S HOSPITAL, INC. The sequence listing filed with the application follows.

SEQUENCE LISTING (167 sequences)

SEQ ID NO: 1 - protein, 107 aa, Artificial Sequence
  source: /note="Description of Artificial Sequence: Synthetic polypeptide"
DIQMTQSPSSLSASVGDRVTITCRTSQDIGNYLNWYQQKPGKAFKLLIYSTSRLHSGVPSRFSGSGSGTDFTLTISSLQPEDFATYYCQQGIILPITFGGGTKVEIK

SEQ ID NO: 2 - protein, 107 aa, Artificial Sequence
  source: /note="Description of Artificial Sequence: Synthetic polypeptide"
DIQMTQSPSSLSASVGDRVTITCRTSQDIGNYLNWYQQKPGKAFKLLIYSTSRLHSGVPSRFSGSGSGTDFTLTISSLQPEDFATYYCQQGIVLPITFGGGTKVEIK

SEQ ID NO: 3 - protein, 107 aa, Artificial Sequence
  source: /note="Description of Artificial Sequence: Synthetic polypeptide"
DIQMTQSPSSLSASVGDRVTITCRTSQDISNYLNWYQQKPGKAFKLLIFSTSRLHSGVPSRFSGSGSGTDFTLTISSLQPEDFATYYCQQGIVLPITFGGGTKVEIK

SEQ ID NO: 4 - protein, 107 aa, Artificial Sequence
  source: /note="Description of Artificial Sequence: Synthetic polypeptide"
DIQMTQSPSSLSASVGDRVTITCRTSQDISSYLNWYQQKPGKAFKLLIYSTSRLHSGVPSRFSGSGSGTDFTLTISSLQPEDFATYYCQQGIVLPITFGGGTKVEIK

SEQ ID NO: 5 - protein, 107 aa, Artificial Sequence
  source: /note="Description of Artificial Sequence: Synthetic polypeptide"
DIQMTQSPSSLSASVGDRVTITCRTSQDISNYLNWYQQKPGKAFKLLIYTTSRLRSGVPSRFSGSGSGTDFTLTISSLQPEDFATYYCQQGIVLPITFGGGTKVEIK

SEQ ID NO: 6 - protein, 107 aa, Artificial Sequence
  source: /note="Description of Artificial Sequence: Synthetic polypeptide"
DIQMTQSPSSLSASVGDRVTITCRTSQDIDNFLQWYQQKPGKAFKLLIYSTSRLHSGVPSRFSGSGSGTDFTLTISSLQPEDFATYYCQQGIVLPITFGGGTKVEIK

SEQ ID NO: 7 - protein, 107 aa, Artificial Sequence
  source: /note="Description of Artificial Sequence: Synthetic polypeptide"
DIQMTQSPSSLSASVGDRVTITCRTSQDISNYLNWYQQKPGKAFKLLIYSTSKLHSGVPSRFSGSGSGTDFTLTISSLQPEDFATYYCQQGIVLPITFGGGTKVEIK

SEQ ID NO: 8 - protein, 107 aa, Artificial Sequence
  source: /note="Description of Artificial Sequence: Synthetic polypeptide"
DIQMTQSPSSLSASVGDRVTITCRTSQDIGNYLNWYQQKPGKAFKLLIYSTSRLHSGVPSRFSGSGSGTDFTLTISSLQPEDFATYYCQQSTILPLTFGGGTKVEIK

SEQ ID NO: 9 - protein, 107 aa, Artificial Sequence
  source: /note="Description of Artificial Sequence: Synthetic polypeptide"
DIQMTQSPSSLSASVGDRVTITCRTSQDISNYLNWYQQKPGKAFKLLIFSTSRLHSGVPSRFSGSGSGTDFTLTISSLQPEDFATYYCQQSTILPLTFGGGTKVEIK

SEQ ID NO: 10 - protein, 107 aa, Artificial Sequence
  source: /note="Description of Artificial Sequence: Synthetic polypeptide"
DIQMTQSPSSLSASVGDRVTITCRTSQDISSYLNWYQQKPGKAFKLLIYSTSRLHSGVPSRFSGSGSGTDFTLTISSLQPEDFATYYCQQSTILPLTFGGGTKVEIK

SEQ ID NO: 11 - protein, 107 aa, Artificial Sequence
  source: /note="Description of Artificial Sequence: Synthetic polypeptide"
DIQMTQSPSSLSASVGDRVTITCRTSQDISNYLNWYQQKPGKAFKLLIYTTSRLRSGVPSRFSGSGSGTDFTLTISSLQPEDFATYYCQQSTILPLTFGGGTKVEIK

SEQ ID NO: 12 - protein, 107 aa, Artificial Sequence
  source: /note="Description of Artificial Sequence: Synthetic polypeptide"
DIQMTQSPSSLSASVGDRVTITCRTSQDIDNFLQWYQQKPGKAFKLLIYSTSRLHSGVPSRFSGSGSGTDFTLTISSLQPEDFATYYCQQSTILPLTFGGGTKVEIK

SEQ ID NO: 13 - protein, 107 aa, Artificial Sequence
  source: /note="Description of Artificial Sequence: Synthetic polypeptide"
DIQMTQSPSSLSASVGDRVTITCRTSQDISNYLNWYQQKPGKAFKLLIYSTSKLHSGVPSRFSGSGSGTDFTLTISSLQPEDFATYYCQQSTILPLTFGGGTKVEIK

SEQ ID NO: 14 - protein, 107 aa, Artificial Sequence
  source: /note="Description of Artificial Sequence: Synthetic polypeptide"
DIQMTQSPSSLSASVGDRVTITCRTSQDISNYLNWYQQKPGKAFKLLIFSTSRLHSGVPSRFSGSGSGTDFTLTISSLQPEDFATYYCQQGIILPITFGGGTKVEIK

SEQ ID NO: 15 - protein, 107 aa, Artificial Sequence
  source: /note="Description of Artificial Sequence: Synthetic polypeptide"
DIQMTQSPSSLSASVGDRVTITCRTSQDISSYLNWYQQKPGKAFKLLIYSTSRLHSGVPSRFSGSGSGTDFTLTISSLQPEDFATYYCQQGIILPITFGGGTKVEIK

SEQ ID NO: 16 - protein, 107 aa, Artificial Sequence
  source: /note="Description of Artificial Sequence: Synthetic polypeptide"
DIQMTQSPSSLSASVGDRVTITCRTSQDISNYLNWYQQKPGKAFKLLIYTTSRLRSGVPSRFSGSGSGTDFTLTISSLQPEDFATYYCQQGIILPITFGGGTKVEIK

SEQ ID NO: 17 - protein, 107 aa, Artificial Sequence
  source: /note="Description of Artificial Sequence: Synthetic polypeptide"
DIQMTQSPSSLSASVGDRVTITCRTSQDIDNFLQWYQQKPGKAFKLLIYSTSRLHSGVPSRFSGSGSGTDFTLTISSLQPEDFATYYCQQGIILPITFGGGTKVEIK

SEQ ID NO: 18 - protein, 107 aa, Artificial Sequence
  source: /note="Description of Artificial Sequence: Synthetic polypeptide"
DIQMTQSPSSLSASVGDRVTITCRTSQDISNYLNWYQQKPGKAFKLLIYSTSKLHSGVPSRFSGSGSGTDFTLTISSLQPEDFATYYCQQGIILPITFGGGTKVEIK

SEQ ID NO: 19 - protein, 107 aa, Artificial Sequence
  source: /note="Description of Artificial Sequence: Synthetic polypeptide"
DIQMTQSPSSLSASVGDRVTITCRTSQDIGNYLNWYQQKPGKAFKLLIFSTSRLHSGVPSRFSGSGSGTDFTLTISSLQPEDFATYYCQQGIVLPITFGGGTKVEIK

SEQ ID NO: 20 - protein, 107 aa, Artificial Sequence
  source: /note="Description of Artificial Sequence: Synthetic polypeptide"
DIQMTQSPSSLSASVGDRVTITCRTSQDISSYLNWYQQKPGKAFKLLIYTTSRLRSGVPSRFSGSGSGTDFTLTISSLQPEDFATYYCQQGIVLPITFGGGTKVEIK

SEQ ID NO: 21 - protein, 107 aa, Artificial Sequence
  source: /note="Description of Artificial Sequence: Synthetic polypeptide"
DIQMTQSPSSLSASVGDRVTITCRTSQDIDNFLQWYQQKPGKAFKLLIFSTSKLHSGVPSRFSGSGSGTDFTLTISSLQPEDFATYYCQQGIVLPITFGGGTKVEIK

SEQ ID NO: 22 - protein, 107 aa, Artificial Sequence
  source: /note="Description of Artificial Sequence: Synthetic polypeptide"
DIQMTQSPSSLSASVGDRVTITCRTSQDIGNYLNWYQQKPGKAFKLLIFSTSRLHSGVPSRFSGSGSGTDFTLTISSLQPEDFATYYCQQSTILPLTFGGGTKVEIK

SEQ ID NO: 23 - protein, 107 aa, Artificial Sequence
  source: /note="Description of Artificial Sequence: Synthetic polypeptide"
DIQMTQSPSSLSASVGDRVTITCRTSQDISSYLNWYQQKPGKAFKLLIYTTSRLRSGVPSRFSGSGSGTDFTLTISSLQPEDFATYYCQQSTILPLTFGGGTKVEIK

SEQ ID NO: 24 - protein, 107 aa, Artificial Sequence
  source: /note="Description of Artificial Sequence: Synthetic polypeptide"
DIQMTQSPSSLSASVGDRVTITCRTSQDIDNFLQWYQQKPGKAFKLLIFSTSKLHSGVPSRFSGSGSGTDFTLTISSLQPEDFATYYCQQSTILPLTFGGGTKVEIK

SEQ ID NO: 25 - protein, 107 aa, Artificial Sequence
  source: /note="Description of Artificial Sequence: Synthetic polypeptide"
DIQMTQSPSSLSASVGDRVTITCRTSQDIGNYLNWYQQKPGKAFKLLIFSTSRLHSGVPSRFSGSGSGTDFTLTISSLQPEDFATYYCQQGIILPITFGGGTKVEIK

SEQ ID NO: 26 - protein, 107 aa, Artificial Sequence
  source: /note="Description of Artificial Sequence: Synthetic polypeptide"
DIQMTQSPSSLSASVGDRVTITCRTSQDISSYLNWYQQKPGKAFKLLIYTTSRLRSGVPSRFSGSGSGTDFTLTISSLQPEDFATYYCQQGIILPITFGGGTKVEIK

SEQ ID NO: 27 - protein, 107 aa, Artificial Sequence
  source: /note="Description of Artificial Sequence: Synthetic polypeptide"
DIQMTQSPSSLSASVGDRVTITCRTSQDIDNFLQWYQQKPGKAFKLLIFSTSKLHSGVPSRFSGSGSGTDFTLTISSLQPEDFATYYCQQGIILPITFGGGTKVEIK

SEQ ID NO: 28 - protein, 119 aa, Artificial Sequence
  source: /note="Description of Artificial Sequence: Synthetic polypeptide"
QVQLVQSGAEVKKPGSSVKVSCKASGYTFSRYWMHWVRQAPGQGLEWMGHIDPSDSYTYYNQKFKGRVTITADESTSTAYMELSSLRSEDTAVYYCARWDYGNLLFEYWGQGTLVTVSS

SEQ ID NO: 29 - protein, 330 aa, Artificial Sequence
  source: /note="Description of Artificial Sequence: Synthetic polypeptide"
  VARIANT (330)..(330): /replace=" "
  MISC_FEATURE (1)..(330): /note="Variant residues given in the sequence have no preference with respect to those in the annotations for variant positions"
ASTKGPSVFPLAPSSKSTSGGTAALGCLVKDYFPEPVTVSWNSGALTSGVHTFPAVLQSSGLYSLSSVVTVPSSSLGTQTYICNVNHKPSNTKVDKKVEPKSCDKTHTCPPCPAPEAAGAPSVFLFPPKPKDTLMISRTPEVTCVVVDVSHEDPEVKFNWYVDGVEVHNAKTKPREEQYNSTYRVVSVLTVLHQDWLNGKEYKCKVSNKALPAPIEKTISKAKGQPREPQVYTLPPSREEMTKNQVSLTCLVKGFYPSDIAVEWESNGQPENNYKTTPPVLDSDGSFFLYSKLTVDKSRWQQGNVFSCSVMHEALHNHYTQKSLSLSPGK

SEQ ID NO: 30 - protein, 107 aa, Artificial Sequence [sequence omitted]

SEQ ID NO: 31 - skipped

SEQ ID NO: 32 - protein, 214 aa, Artificial Sequence
  source: /note="Description of Artificial Sequence: Synthetic polypeptide"
DIQMTQSPSSLSASVGDRVTITCRTSQDIGNYLNWYQQKPGKAFKLLIYSTSRLHSGVPSRFSGSGSGTDFTLTISSLQPEDFATYYCQQGIILPITFGGGTKVEIKRTVAAPSVFIFPPSDEQLKSGTASVVCLLNNFYPREAKVQWKVDNALQSGNSQESVTEQDSKDSTYSLSSTLTLSKADYEKHKVYACEVTHQGLSSPVTKSFNRGEC

SEQ ID NO: 33 - protein, 449 aa, Artificial Sequence
  source: /note="Description of Artificial Sequence: Synthetic polypeptide"
  VARIANT (449)..(449): /replace=" "
  MISC_FEATURE (1)..(449): /note="Variant residues given in the sequence have no preference with respect to those in the annotations for variant positions"
QVQLVQSGAEVKKPGSSVKVSCKASGYTFSRYWMHWVRQAPGQGLEWMGHIDPSDSYTYYNQKFKGRVTITADESTSTAYMELSSLRSEDTAVYYCARWDYGNLLFEYWGQGTLVTVSSASTKGPSVFPLAPSSKSTSGGTAALGCLVKDYFPEPVTVSWNSGALTSGVHTFPAVLQSSGLYSLSSVVTVPSSSLGTQTYICNVNHKPSNTKVDKKVEPKSCDKTHTCPPCPAPEAAGAPSVFLFPPKPKDTLMISRTPEVTCVVVDVSHEDPEVKFNWYVDGVEVHNAKTKPREEQYNSTYRVVSVLTVLHQDWLNGKEYKCKVSNKALPAPIEKTISKAKGQPREPQVYTLPPSREEMTKNQVSLTCLVKGFYPSDIAVEWESNGQPENNYKTTPPVLDSDGSFFLYSKLTVDKSRWQQGNVFSCSVMHEALHNHYTQKSLSLSPGK

SEQ ID NO: 34 - protein, 11 aa, Artificial Sequence
  source: /note="Description of Artificial Sequence: Synthetic peptide"
RTSQDIGNYLN

SEQ ID NO: 35 - protein, 7 aa, Artificial Sequence
  source: /note="Description of Artificial Sequence: Synthetic peptide"
STSRLHS

SEQ ID NO: 36 - protein, 9 aa, Artificial Sequence
  source: /note="Description of Artificial Sequence: Synthetic peptide"
QQGIILPIT

SEQ ID NO: 37 - protein, 10 aa, Artificial Sequence
  source: /note="Description of Artificial Sequence: Synthetic peptide"
GYTFSRYWMH

SEQ ID NO: 38 - protein, 17 aa, Artificial Sequence
  source: /note="Description of Artificial Sequence: Synthetic peptide"
HIDPSDSYTYYNQKFKG

SEQ ID NO: 39 - protein, 10 aa, Artificial Sequence
  source: /note="Description of Artificial Sequence: Synthetic peptide"
WDYGNLLFEY

SEQ ID NO: 40 - protein, 187 aa, Homo sapiens
MTNKCLLQIALLLCFSTTALSMSYNLLGFLQRSSNFQCQKLLWQLNGRLEYCLKDRMNFDIPEEIKQLQQFQKEDAALTIYEMLQNIFAIFRQDSSSTGWNETIVENLLANVYHQINHLKTVLEEKLEKEDFTRGKLMSSLHLKRYYGRILHYLKAKEYSHCAWTIVRVEILRNFYFINRLTGYLRN

SEQ ID NO: 41 - protein, 166 aa, Homo sapiens
MSYNLLGFLQRSSNFQCQKLLWQLNGRLEYCLKDRMNFDIPEEIKQLQQFQKEDAALTIYEMLQNIFAIFRQDSSSTGWNETIVENLLANVYHQINHLKTVLEEKLEKEDFTRGKLMSSLHLKRYYGRILHYLKAKEYSHCAWTIVRVEILRNFYFINRLTGYLRN

SEQ ID NO: 42 - protein, 161 aa, Mus sp.
INYKQLQLQERTNIRKCQELLEQLNGKINLTYRADFKIPMEMTEKMQKSYTAFAIQEMLQNVFLVFRNNFSSTGWNETIVVRLLDELHQQTVFLKTVLEEKQEERLTWEMSSTALHLKSYYWRVQRYLKLMKYNSYAWMVVRAEIFRNFLIIRRLTRNFQN

SEQ ID NO: 43 - protein, 163 aa, Rattus sp.
IDYKQLQFRQSTSIRTCQKLLRQLNGRLNLSYRTDFKIPMEVMHPSQMEKSYTAFAIQVMLQNVFLVFRSNFSSTGWNETIVESLLDELHQQTELLEIILKEKQEERLTWVTSTTTLGLKSYYWRVQRYLKDKKYNSYAWMVVRAEVFRNFSIILRLNRNFQN

SEQ ID NO: 44 - protein, 166 aa, Macaca fascicularis
MSYNLLGFLQRSSSFQCQKLLWQLNGRLEYCLKDRMNFDIPEEIKQPQQFQKEDAALTIYEMLQNIYAIFRQDLSSTGWNETIVENLLANVYHQIDHLKTILEEKLEKEDFTRGKFVSSLHLKRYYGRILHYLKAKEYSHCAWTIVRVEILRNFFFINKLTGYLRN

SEQ ID NO: 45 - protein, 159 aa, Oryctolagus cuniculus
MSYNSLQIQLWHGSLTCAKLLLQLNGTTEDCLNERINFKVPKEIKEPQQLQKEDTTLVIFEMLNNIFDIFRKNFSSTGWNETLVENLLGETHLQIHHLKSKINKKVTLESIRMNLRLKSYYWRIMDYLETKQYSNCAWKIVQLEIFRNFSFIIMLIDYL

SEQ ID NO: 46 - protein, 11 aa, Artificial Sequence
  source: /note="Description of Artificial Sequence: Synthetic peptide"
RASQSISSYLN

SEQ ID NO: 47 - protein, 7 aa, Artificial Sequence
  source: /note="Description of Artificial Sequence: Synthetic peptide"
AASSLQS

SEQ ID NO: 48 - protein, 7 aa, Artificial Sequence
  source: /note="Description of Artificial Sequence: Synthetic peptide"
QQSYSTP

SEQ ID NO: 49 - protein, 16 aa, Artificial Sequence
  source: /note="Description of Artificial Sequence: Synthetic peptide"
KSSQSLLHSDGKTYLY

SEQ ID NO: 50 - protein, 7 aa, Artificial Sequence
  source: /note="Description of Artificial Sequence: Synthetic peptide"
EVSNRFS

SEQ ID NO: 51 - protein, 7 aa, Artificial Sequence
  source: /note="Description of Artificial Sequence: Synthetic peptide"
MQSIQLP

SEQ ID NO: 52 - protein, 16 aa, Artificial Sequence
  source: /note="Description of Artificial Sequence: Synthetic peptide"
RSSQSLVYSDGNTYLN

SEQ ID NO: 53 - protein, 7 aa, Artificial Sequence
  source: /note="Description of Artificial Sequence: Synthetic peptide"
KVSNRDS

SEQ ID NO: 54 - protein, 7 aa, Artificial Sequence
  source: /note="Description of Artificial Sequence: Synthetic peptide"
MQGTHWP

SEQ ID NO: 55 - protein, 17 aa, Artificial Sequence
  source: /note="Description of Artificial Sequence: Synthetic peptide"
KSSQSVLYSSNNKNYLA

SEQ ID NO: 56 - protein, 7 aa, Artificial Sequence
  source: /note="Description of Artificial Sequence: Synthetic peptide"
WASTRES

SEQ ID NO: 57 - protein, 7 aa, Artificial Sequence
  source: /note="Description of Artificial Sequence: Synthetic peptide"
QQYYSTP

SEQ ID NO: 58 - protein, 11 aa, Artificial Sequence
  source: /note="Description of Artificial Sequence: Synthetic peptide"
RASQSISSWLA

SEQ ID NO: 59 - protein, 7 aa, Artificial Sequence
  source: /note="Description of Artificial Sequence: Synthetic peptide"
DASSLES

SEQ ID NO: 60 - protein, 7 aa, Artificial Sequence
  source: /note="Description of Artificial Sequence: Synthetic peptide"
QQYNSYS

SEQ ID NO: 61 - protein, 11 aa, Artificial Sequence
  source: /note="Description of Artificial Sequence: Synthetic peptide"
QASQDISNYLN

SEQ ID NO: 62 - protein, 7 aa, Artificial Sequence
  source: /note="Description of Artificial Sequence: Synthetic peptide"
DASNLET

SEQ ID NO: 63 - protein, 7 aa, Artificial Sequence
  source: /note="Description of Artificial Sequence: Synthetic peptide"
QQYDNLP

SEQ ID NO: 64 - protein, 11 aa, Artificial Sequence
  source: /note="Description of Artificial Sequence: Synthetic peptide"
RASQGISSYLA

SEQ ID NO: 65 - protein, 7 aa, Artificial Sequence
  source: /note="Description of Artificial Sequence: Synthetic peptide"
AASTLQS

SEQ ID NO: 66 - protein, 7 aa, Artificial Sequence
  source: /note="Description of Artificial Sequence: Synthetic peptide"
QQLNSYP

SEQ ID NO: 67 - protein, 11 aa, Artificial Sequence
  source: /note="Description of Artificial Sequence: Synthetic peptide"
RASQSVSSNLA

SEQ ID NO: 68 - protein, 7 aa, Artificial Sequence
  source: /note="Description of Artificial Sequence: Synthetic peptide"
GASTRAT

SEQ ID NO: 69 - protein, 7 aa, Artificial Sequence
  source: /note="Description of Artificial Sequence: Synthetic peptide"
QQYNNWP

SEQ ID NO: 70 - protein, 11 aa, Artificial Sequence
  source: /note="Description of Artificial Sequence: Synthetic peptide"
RASQSVSSYLA

SEQ ID NO: 71 - protein, 7 aa, Artificial Sequence
  source: /note="Description of Artificial Sequence: Synthetic peptide"
DASNRAT

SEQ ID NO: 72 - protein, 7 aa, Artificial Sequence
  source: /note="Description of Artificial Sequence: Synthetic peptide"
QQRSNWP

SEQ ID NO: 73 - protein, 12 aa, Artificial Sequence
  source: /note="Description of Artificial Sequence: Synthetic peptide"
RASQSVSSSYLA

SEQ ID NO: 74 - protein, 7 aa, Artificial Sequence
  source: /note="Description of Artificial Sequence: Synthetic peptide"
GASSRAT

SEQ ID NO: 75 - protein, 7 aa, Artificial Sequence
  source: /note="Description of Artificial Sequence: Synthetic peptide"
QQYGSSP

SEQ ID NO: 76 - protein, 16 aa, Artificial Sequence
  source: /note="Description of Artificial Sequence: Synthetic peptide"
RSSQSLLHSNGYNYLD

SEQ ID NO: 77 - protein, 7 aa, Artificial Sequence
  source: /note="Description of Artificial Sequence: Synthetic peptide"
LGSNRAS

SEQ ID NO: 78 - protein, 7 aa, Artificial Sequence
  source: /note="Description of Artificial Sequence: Synthetic peptide"
MQALQTP

SEQ ID NO: 79 - protein, 11 aa, Artificial Sequence
  source: /note="Description of Artificial Sequence: Synthetic peptide"
QGDSLRSYYAS

SEQ ID NO: 80 - protein, 7 aa, Artificial Sequence
  source: /note="Description of Artificial Sequence: Synthetic peptide"
GKNNRPS

SEQ ID NO: 81 - protein, 9 aa, Artificial Sequence
  source: /note="Description of Artificial Sequence: Synthetic peptide"
NSRDSSGNH

SEQ ID NO: 82 - protein, 14 aa, Artificial Sequence
  source: /note="Description of Artificial Sequence: Synthetic peptide"
TGSSSNIGAGYDVH

SEQ ID NO: 83 - protein, 7 aa, Artificial Sequence
  source: /note="Description of Artificial Sequence: Synthetic peptide"
GNSNRPS

SEQ ID NO: 84 - protein, 9 aa, Artificial Sequence
  source: /note="Description of Artificial Sequence: Synthetic peptide"
QSYDSSLSG

SEQ ID NO: 85 - protein, 13 aa, Artificial Sequence
  source: /note="Description of Artificial Sequence: Synthetic peptide"
TRSSGSIASNYVQ

SEQ ID NO: 86 - protein, 7 aa, Artificial Sequence
  source: /note="Description of Artificial Sequence: Synthetic peptide"
EDNQRPS

SEQ ID NO: 87 - protein, 7 aa, Artificial Sequence
  source: /note="Description of Artificial Sequence: Synthetic peptide"
QSYDSSN

SEQ ID NO: 88 - protein, 12 aa, Artificial Sequence
  source: /note="Description of Artificial Sequence: Synthetic peptide"
TGSSSGGSYYVS

SEQ ID NO: 89 - protein, 14 aa, Artificial Sequence
  source: /note="Description of Artificial Sequence: Synthetic peptide"
TGSSSDVGGSYYVS

SEQ ID NO: 90 - protein, 8 aa, Artificial Sequence
  source: /note="Description of Artificial Sequence: Synthetic peptide"
ENDSNRPS

SEQ ID NO: 91 - protein, 12 aa, Artificial Sequence
  source: /note="Description of Artificial Sequence: Synthetic peptide"
  VARIANT (6)..(6): /replace="Asp"
  VARIANT (8)..(8): /replace="Gly"
  MISC_FEATURE (1)..(12): /note="Variant residues given in the sequence have no preference with respect to those in the annotations for variant positions"
EDSNRSKQQKPS

SEQ ID NO: 92 - protein, 8 aa, Artificial Sequence
  source: /note="Description of Artificial Sequence: Synthetic peptide"
  VARIANT (8)..(8): /replace="Thr"
  MISC_FEATURE (1)..(8): /note="Variant residues given in the sequence have no preference with respect to those in the annotations for variant positions"
QSWDSSAN

SEQ ID NO: 93 - protein, 11 aa, Artificial Sequence
  source: /note="Description of Artificial Sequence: Synthetic peptide"
  VARIANT (8)..(8): /replace="Thr"
  VARIANT (10)..(10): /replace="Val"
  VARIANT (11)..(11): /replace="Val"
  MISC_FEATURE (1)..(11): /note="Variant residues given in the sequence have no preference with respect to those in the annotations for variant positions"
QSWDSSANFFG

SEQ ID NO: 94 - protein, 13 aa, Artificial Sequence
  source: /note="Description of Artificial Sequence: Synthetic peptide"
  VARIANT (11)..(11): /replace="Tyr"
  VARIANT (13)..(13): /replace="His" or "Ser"
  MISC_FEATURE (1)..(13): /note="Variant residues given in the sequence have no preference with respect to those in the annotations for variant positions"
SGSSSNIGNNAVN

SEQ ID NO: 95 - protein, 14 aa, Artificial Sequence
  source: /note="Description of Artificial Sequence: Synthetic peptide"
  VARIANT (12)..(12): /replace="Tyr"
  VARIANT (14)..(14): /replace="His" or "Ser"
  MISC_FEATURE (1)..(14): /note="Variant residues given in the sequence have no preference with respect to those in the annotations for variant positions"
SGSSSNIIGNNAVN

SEQ ID NO: 96 - protein, 7 aa, Artificial Sequence
  source: /note="Description of Artificial Sequence: Synthetic peptide"
  VARIANT (4)..(4): /replace="Asn" or "Gln"
  MISC_FEATURE (1)..(7): /note="Variant residues given in the sequence have no preference with respect to those in the annotations for variant positions"
GNNKRPS

SEQ ID NO: 97 - protein, 9 aa, Artificial Sequence
  source: /note="Description of Artificial Sequence: Synthetic peptide"
  VARIANT (8)..(8): /replace="Ser"
  MISC_FEATURE (1)..(9): /note="Variant residues given in the sequence have no preference with respect to those in the annotations for variant positions"
AAWDDSLNG

SEQ ID NO: 98 - protein, 12 aa, Artificial Sequence
  source: /note="Description of Artificial Sequence: Synthetic peptide"
  VARIANT (5)..(5): /replace="Val"
  VARIANT (8)..(8): /replace="Ser"
  MISC_FEATURE (1)..(12): /note="Variant residues given in the sequence have no preference with respect to those in the annotations for variant positions"
CSGDALGKKYAH

SEQ ID NO: 99 - protein, 7 aa, Artificial Sequence
  source: /note="Description of Artificial Sequence: Synthetic peptide"
KDSERPS

SEQ ID NO: 100 - protein, 8 aa, Artificial Sequence
  source: /note="Description of Artificial Sequence: Synthetic peptide"
  VARIANT (8)..(8): /replace="Asp" or "Thr" or "Ala"
  MISC_FEATURE (1)..(8): /note="Variant residues given in the sequence have no preference with respect to those in the annotations for variant positions"
QSWDSSGN

SEQ ID NO: 101 - protein, 9 aa, Artificial Sequence
  source: /note="Description of Artificial Sequence: Synthetic peptide"
  VARIANT (8)..(8): /replace="Asp" or "Thr" or "Ala"
  MISC_FEATURE (1)..(9): /note="Variant residues given in the sequence have no preference with respect to those in the annotations for variant positions"
QSWDSSGNH

SEQ ID NO: 102 - protein, 17 aa, Artificial Sequence
  source: /note="Description of Artificial Sequence: Synthetic peptide"
RASQSLLHSDGISSYLA

SEQ ID NO: 103 - protein, 11 aa, Artificial Sequence
  source: /note="Description of Artificial Sequence: Synthetic peptide"
RASQGISSYLA

SEQ ID NO: 104 - protein, 7 aa, Artificial Sequence
  source: /note="Description of Artificial Sequence: Synthetic peptide"
AASSRAS

SEQ ID NO: 105 - protein, 7 aa, Artificial Sequence
  source: /note="Description of Artificial Sequence: Synthetic peptide"
QQYNSYP

SEQ ID NO: 106 - protein, 11 aa, Artificial Sequence
  source: /note="Description of Artificial Sequence: Synthetic peptide"
  VARIANT (8)..(8): /replace="Ser"
  MISC_FEATURE (1)..(11): /note="Variant residues given in the sequence have no preference with respect to those in the annotations for variant positions"
RASQGISNYLA

SEQ ID NO: 107 - protein, 7 aa, Artificial Sequence
  source: /note="Description of Artificial Sequence: Synthetic peptide"
AASSLQS

SEQ ID NO: 108 - protein, 7 aa, Artificial Sequence
  source: /note="Description of Artificial Sequence: Synthetic peptide"
QQYNSYP

SEQ ID NO: 109 - protein, 16 aa, Artificial Sequence
  source: /note="Description of Artificial Sequence: Synthetic peptide"
RSSQSLLHSDGNTYLD

SEQ ID NO: 110 - protein, 17 aa, Artificial Sequence
  source: /note="Description of Artificial Sequence: Synthetic peptide"
RSSQSLLHSDDGNTYLD

SEQ ID NO: 111 - protein, 7 aa, Artificial Sequence
  source: /note="Description of Artificial Sequence: Synthetic peptide"
  VARIANT (1)..(1): /replace="Thr"
  VARIANT (2)..(2): /replace="Ile"
  VARIANT (6)..(6): /replace="Phe"
  MISC_FEATURE (1)..(7): /note="Variant residues given in the sequence have no preference with respect to those in the annotations for variant positions"
KVSNRAS

SEQ ID NO: 112 - protein, 7 aa, Artificial Sequence
  source: /note="Description of Artificial Sequence: Synthetic peptide"
MQATQFP

SEQ ID NO: 113 - protein, 12 aa, Artificial Sequence
  source: /note="Description of Artificial Sequence: Synthetic peptide"
  VARIANT (6)..(7): /replace="Val"
  MISC_FEATURE (1)..(12): /note="Variant residues given in the sequence have no preference with respect to those in the annotations for variant positions"
RASQSSSSSYLA

SEQ ID NO: 114 - protein, 7 aa, Artificial Sequence
  source: /note="Description of Artificial Sequence: Synthetic peptide"
GASTRAT

SEQ ID NO: 115 - protein, 7 aa, Artificial Sequence
  source: /note="Description of Artificial Sequence: Synthetic peptide"
  VARIANT (4)..(4): /replace="Asn" or "Gly" or "His"
  MISC_FEATURE (1)..(7): /note="Variant residues given in the sequence have no preference with respect to those in the annotations for variant positions"
QQYSNWP

SEQ ID NO: 116 - protein, 10 aa, Artificial Sequence
  source: /note="Description of Artificial Sequence: Synthetic peptide"
GFTFSSYWMS

SEQ ID NO: 117 - protein, 18 aa, Artificial Sequence
  source: /note="Description of Artificial Sequence: Synthetic peptide"
ANIKQDGSEKYYVDSVKG

SEQ ID NO: 118 - protein, 10 aa, Artificial Sequence
  source: /note="Description of Artificial Sequence: Synthetic peptide"
GFTFSSYAMS

SEQ ID NO: 119 - protein, 17 aa, Artificial Sequence
  source: /note="Description of Artificial Sequence: Synthetic peptide"
AISGSGGSTYYADSVKG

SEQ ID NO: 120 - protein, 10 aa, Artificial Sequence
  source: /note="Description of Artificial Sequence: Synthetic peptide"
GGSISSYYWS

SEQ ID NO: 121 - protein, 17 aa, Artificial Sequence
  source: /note="Description of Artificial Sequence: Synthetic peptide"
GYIYYSGSTNYNPSLKS

SEQ ID NO: 122 - protein, 10 aa, Artificial Sequence
  source: /note="Description of Artificial Sequence: Synthetic peptide"
GYTFTGYYMH

SEQ ID NO: 123 - protein, 18 aa, Artificial Sequence
  source: /note="Description of Artificial Sequence: Synthetic peptide"
GWINPNSGGTNYAQKFQG

SEQ ID NO: 124 - protein, 10 aa, Artificial Sequence
  source: /note="Description of Artificial Sequence: Synthetic peptide"
GGTFSSYAIS

SEQ ID NO: 125 - protein, 18 aa, Artificial Sequence
  source: /note="Description of Artificial Sequence: Synthetic peptide"
GGIIPIFGTANYAQKFQG

SEQ ID NO: 126 - protein, 10 aa, Artificial Sequence
  source: /note="Description of Artificial Sequence: Synthetic peptide"
GYTGTSYYMH

SEQ ID NO: 127 - protein, 18 aa, Artificial Sequence
  source: /note="Description of Artificial Sequence: Synthetic peptide"
GIINPSGGSTSYAQKFQG

SEQ ID NO: 128 - protein, 10 aa, Artificial Sequence
  source: /note="Description of Artificial Sequence: Synthetic peptide"
GFTFSSYGMH

SEQ ID NO: 129 - protein, 18 aa, Artificial Sequence
  source: /note="Description of Artificial Sequence: Synthetic peptide"
AVISYDGSNKYYADSVKG

SEQ ID NO: 130 - protein, 10 aa, Artificial Sequence
  source: /note="Description of Artificial Sequence: Synthetic peptide"
GFTFSSYSMN

SEQ ID NO: 131 - protein, 18 aa, Artificial Sequence
  source: /note="Description of Artificial Sequence: Synthetic peptide"
SYISSSSSTIYYADSVKG

SEQ ID NO: 132 - protein, 10 aa, Artificial Sequence
  source: /note="Description of Artificial Sequence: Synthetic peptide"
GFTFSNAWMS

SEQ ID NO: 133 - protein, 20 aa, Artificial Sequence
  source: /note="Description of Artificial Sequence: Synthetic peptide"
GRIKSKTDGGTTDYAAPVKG

SEQ ID NO: 134 - protein, 12 aa, Artificial Sequence
  source: /note="Description of Artificial Sequence: Synthetic peptide"
GGSISSSSYYWG

SEQ ID NO: 135 - protein, 17 aa, Artificial Sequence
  source: /note="Description of Artificial Sequence: Synthetic peptide"
GSIYYSGSTYYNPSLKS

SEQ ID NO: 136 - protein, 12 aa, Artificial Sequence
  source: /note="Description of Artificial Sequence: Synthetic peptide"
GGSISSGDYYWS

SEQ ID NO: 137 - protein, 17 aa, Artificial Sequence
  source: /note="Description of Artificial Sequence: Synthetic peptide"
GYIYYSGSTYYNPSLKS

SEQ ID NO: 138 - protein, 10 aa, Artificial Sequence
  source: /note="Description of Artificial Sequence: Synthetic peptide"
GYSFTSYWIG

SEQ ID NO: 139 - protein, 18 aa, Artificial Sequence
  source: /note="Description of Artificial Sequence: Synthetic peptide"
GIIYPGDSDTRYSPSFQG

SEQ ID NO: 140 - protein, 10 aa, Artificial Sequence
  source: /note="Description of Artificial Sequence: Synthetic peptide"
  VARIANT (10)..(10): /replace="Ser"
  MISC_FEATURE (1)..(10): /note="Variant residues given in the sequence have no preference with respect to those in the annotations for variant positions"
GFTFSSYAMH

SEQ ID NO: 141 - protein, 12 aa, Artificial Sequence
  source: /note="Description of Artificial Sequence: Synthetic peptide"
  VARIANT (10)..(10): /replace="Ser"
  MISC_FEATURE (1)..(12): /note="Variant residues given in the sequence have no preference with respect to those in the annotations for variant positions"
GFTFSSYAMHWS

SEQ ID NO: 142 - protein, 18 aa, Artificial Sequence
  source: /note="Description of Artificial Sequence: Synthetic peptide"
GWISPNGGSTYYADSVKG

SEQ ID NO: 143 - protein, 20 aa, Artificial Sequence
  source: /note="Description of Artificial Sequence: Synthetic peptide"
GWISPKANGGSTYYADSVKG

SEQ ID NO: 144 - protein, 10 aa, Artificial Sequence
  source: /note="Description of Artificial Sequence: Synthetic peptide"
GFTFSSYAMS

SEQ ID NO: 145 - protein, 18 aa, Artificial Sequence
  source: /note="Description of Artificial Sequence: Synthetic peptide"
  VARIANT (8)..(8): /replace="Ser"
  MISC_FEATURE (1)..(18): /note="Variant residues given in the sequence have no preference with respect to those in the annotations for variant positions"
SVISSDGGSTYYADSVKG

SEQ ID NO: 146 - protein, 20 aa, Artificial Sequence
  source: /note="Description of Artificial Sequence: Synthetic peptide"
  VARIANT (10)..(10): /replace="Ser"
  MISC_FEATURE (1)..(20): /note="Variant residues given in the sequence have no preference with respect to those in the annotations for variant positions"
SVISSKADGGSTYYADSVKG

SEQ ID NO: 147 - protein, 10 aa, Artificial Sequence
  source: /note="Description of Artificial Sequence: Synthetic peptide"
  VARIANT (10)..(10): /replace="Gly" or "His"
  MISC_FEATURE (1)..(10): /note="Variant residues given in the sequence have no preference with respect to those in the annotations for variant positions"
GYSFTSYWIS

SEQ ID NO: 148 - protein, 18 aa, Artificial Sequence
  source: /note="Description of Artificial Sequence: Synthetic peptide"
  VARIANT (2)..(2): /replace="Ile" or "Ser"
  MISC_FEATURE (1)..(18): /note="Variant residues given in the sequence have no preference with respect to those in the annotations for variant positions"
GRIYPGDSDTRYSPSFQG

SEQ ID NO: 149 - protein, 10 aa, Artificial Sequence
  source: /note="Description of Artificial Sequence: Synthetic peptide"
  VARIANT (8)..(8): /replace="Tyr"
  VARIANT (9)..(9): /replace="Met"
  MISC_FEATURE (1)..(10): /note="Variant residues given in the sequence have no preference with respect to those in the annotations for variant positions"
GYTFTSYAIH

SEQ ID NO: 150 - protein, 17 aa, Artificial Sequence
  source: /note="Description of Artificial Sequence: Synthetic peptide"
  VARIANT (6)..(6): /replace="Tyr"
  MISC_FEATURE (1)..(17): /note="Variant residues given in the sequence have no preference with respect to those in the annotations for variant positions"
GWINPGNGNTNYAQKFQ

SEQ ID NO: 151 - protein, 12 aa, Artificial Sequence
  source: /note="Description of Artificial Sequence: Synthetic peptide"
  VARIANT (8)..(8): /replace="Tyr"
  MISC_FEATURE (1)..(12): /note="Variant residues given in the sequence have no preference with respect to those in the annotations for variant positions"
GGSISSGNYYWS

SEQ ID NO: 152 - protein, 17 aa, Artificial Sequence
  source: /note="Description of Artificial Sequence: Synthetic peptide"
GYIYYSGSTYYNPSLKS

SEQ ID NO: 153 - protein, 19 aa, Homo sapiens
YNLLGFLQRSSNFQCQKLL

SEQ ID NO: 154 - protein, 19 aa, Homo sapiens
KEDAALTIYEMLQNIFAIF

SEQ ID NO: 155 - protein, 26 aa, Homo sapiens
ETIVENLLANVYHQINHLKTVLEEKL

SEQ ID NO: 156 - protein, 17 aa, Homo sapiens
SLHLKRYYGRILHYLKA

SEQ ID NO: 157 - protein, 22 aa, Homo sapiens
HCAWTIVRVEILRNFYFINRLT

SEQ ID NO: 158 - protein, 166 aa, Artificial Sequence
  source: /note="Description of Artificial Sequence: Synthetic polypeptide"
MSYNLLGFLQRSSNRRCLMLLAQLNGRLEYCLKDRMNFDIPEEIKQLQQFQKEDAALTIYEMLQNIFAIFRQDSSSTGWNETIVENLLANVYHQINHLKTVLEEKLEKEDFTRGKLMSSLHLKRYYGRILHYLKAKEYSHCAWTIVRVEILRNFYFINRLTGYLRN

SEQ ID NO: 159 - protein, 166 aa, Artificial Sequence
  source: /note="Description of Artificial Sequence: Synthetic polypeptide"
MSYNLLGFLQRSSNFQCQKLLWQLNGRLEYCLKDRHDFGIPQEIKQLQQFQKEDAALTIYEMLQNIFAIFRQDSSSTGWNETIVENLLANVYHQINHLKTVLEEKLEKEDFTRGKLMSSLHLKRYYGRILHYLKAKEYSHCAWTIVRVEILRNFYFINRLTGYLRN

SEQ ID NO: 160 - protein, 166 aa, Artificial Sequence
  source: /note="Description of Artificial Sequence: Synthetic polypeptide"
MSYNLLGFLQRSSNFQCQKLLWQLNGRLEYCLKDRMNFDIPEEIKQLQQFQKEDAALTIYEMLQNIFAIFRQDSSSTGWNETIVDKLLTNVYHQINHLKTVLEEKLEKEDFTRGKLMSSLHLKRYYGRILHYLKAKEYSHCAWTIVRVEILRNFYFINRLTGYLRN

SEQ ID NO: 161 - protein, 166 aa, Artificial Sequence
  source: /note="Description of Artificial Sequence: Synthetic polypeptide"
MSYNLLGFLQRSSNFQCQKLLWQLNGRLEYCLKDRMNFDIPEEIKQLQQFQKEDAALTIYEMLQNIFAIFRQDSSSTGWNETIVENLLAEVYQQINDLEAVLEEKLEKEDFTRGKLMSSLHLKRYYGRILHYLKAKEYSHCAWTIVRVEILRNFYFINRLTGYLRN

SEQ ID NO: 162 - protein, 166 aa, Artificial Sequence
  source: /note="Description of Artificial Sequence: Synthetic polypeptide"
MSYNLLGFLQRSSNFQCQKLLWQLNGRLEYCLKDRMNFDIPEEIKQLQQFQKEDAALTIYEMLQNIFAIFRQDSSSTGWNETIVENLLANVYHQINHLKTVLEEKLEKEDFTRGKLMSILHLRKYYGRILHYLKAKEYSHCAWTIVRVEILRNFYFINRLTGYLRN

SEQ ID NO: 163 - protein, 166 aa, Artificial Sequence
  source: /note="Description of Artificial Sequence: Synthetic polypeptide"
MSYNLLGFLQRSSNFQCQKLLWQLNGRLEYCLKDRMNFDIPEEIKQLQQFQKEDAALTIYEMLQNIFAIFRQDSSSTGWNETIVENLLANVYHQINHLKTVLEEKLEKEDFTRGKLMSSLHLKRYYGRILHYLKEKKYSHCAWTIVRVEILRNFYFINRLTGYLRN

SEQ ID NO: 164 - protein, 166 aa, Artificial Sequence
  source: /note="Description of Artificial Sequence: Synthetic polypeptide"
MSYNLLGFLQRSSNFQCQKLLWQLNGRLEYCLKDRMNFDIPEEIKQLQQFQKEDAALTIYEMLQNIFAIFRQDSSSTGWNETIVENLLANVYHQINHLKTVLEEKLEKEDFTRGKLMSSLHLKRYYGRILHYLKAKEYSPCAWTIVRVEILRNFYFINRLTGYLRN

SEQ ID NO: 165 - protein, 166 aa, Artificial Sequence
  source: /note="Description of Artificial Sequence: Synthetic polypeptide"
MSYNLLGFLQRSSNFQCQKLLWQLNGRLEYCLKDRMNFDIPEEIKQLQQFQKEDAALTIYEMLQNIFAIFRQDSSSTGWNETIVENLLANVYHQINHLKTVLEEKLEKEDFTRGKLMSSLHLKRYYGRILHYLKAKEYSHCAWTIVRAEILRNFSLITRLTGYLRN

SEQ ID NO: 166 - DNA, 357 bp, Artificial Sequence
  source: /note="Description of Artificial Sequence: Synthetic polynucleotide"
caggtgcagctggtgcagagcggcgccgaggtgaagaagcccggcagcagcgtgaaggtgagctgcaaggccagcggctacaccttcagccggtactggatgcactgggtgcggcaggcccccggccagggcctggagtggatgggccacatcgaccccagcgacagctacacctactacaaccagaagttcaagggccgggtgaccatcaccgccgacgagagcaccagcaccgcctacatggagctgagcagcctgcggagcgaggacaccgccgtgtactactgcgcccggtgggactacggcaacctgctgttcgagtactggggccagggcaccctggtgaccgtctcgagc

SEQ ID NO: 167 - DNA, 321 bp, Artificial Sequence
  source: /note="Description of Artificial Sequence: Synthetic polynucleotide"
gacatccagatgacccagagccccagcagcctgagcgccagcgtgggcgaccgggtgaccatcacctgccggaccagccaggacatcggcaactacctgaactggtaccagcagaagcccggcaaggccttcaagctgctgatctacagcaccagccggctgcacagcggcgtgcccagccggttcagcggcagcggcagcggcaccgacttcaccctgaccatcagcagcctgcagcccgaggacttcgccacctactactgccagcaggggattattttgcccattaccttcggcggcggcaccaaggtggagatcaag